European Patent Specification EP 3 515 931 B1, published May 1, 2024. Title: METHODS FOR ENZYMATIC PEPTIDE LIGATION. Applicant: Nanyang Technological University. The sequence listing filed with the application follows.

SEQUENCE LISTING (17 sequences)

SEQ ID NO: 1 - protein, 474 aa, Ovaloparmena affinis
MVRYLAGAVLLLVVLSVAAAVSGARDGDYLHLPSEVSRFFRPQETNDDHGEDSVGTRWAVLIAGSKGYANYRHQAGVCHAYQILKRGGLKDENIVVFMYDDIAYNESNPRPGVIINSPHGSDVYAGVPKDYTGEEVNAKNFLAAILGNKSAITGGSGKVVDSGPNDHIFIYYTDHGAAGVIGMPSKPYLYADELNDALKKKHASGTYKSLVFYLEACESGSMFEGILPEDLNIYALTSTNTTESSWAYYCPAQENPPPPEYNVCLGDLFSVAWLEDSDVQNSWYETLNQQYHHVDKRISHASHATQYGNLKLGEEGLFVYMGSNPANDNYTSLDGNALTPSSIVVNQRDADLLHLWEKFRKAPEGSARKEEAQTQIFKAMSHRVHIDSSIKLIGKLLFGIEKCTEILNAVRPAGQPLVDDWACLRSLVGTFETHCGSLSEYGMRHTRTIANICNAGISEEQMAEAASQACASIP

SEQ ID NO: 2 - protein, 18 aa, Ovaloparmena affinis
  MISC_FEATURE (1)..(1): Xaa corresponds to position 247 of SEQ ID NO:1 and is Gly, Ala, Ser, or Cys.
  MISC_FEATURE (2)..(2): Xaa is any amino acid, preferably any amino acid that does not disrupt the structural fold of the remaining conserved amino acids
  MISC_FEATURE (6)..(6): Xaa is any amino acid, preferably any amino acid that does not disrupt the structural fold of the remaining conserved amino acids
  MISC_FEATURE (7)..(7): Xaa is any amino acid, preferably any amino acid that does not disrupt the structural fold of the remaining conserved amino acids
  MISC_FEATURE (8)..(8): Xaa is any amino acid, preferably any amino acid that does not disrupt the structural fold of the remaining conserved amino acids
  MISC_FEATURE (9)..(9): Xaa is any amino acid, preferably any amino acid that does not disrupt the structural fold of the remaining conserved amino acids
  MISC_FEATURE (10)..(10): Xaa is any amino acid, preferably any amino acid that does not disrupt the structural fold of the remaining conserved amino acids
  MISC_FEATURE (16)..(16): Xaa is any amino acid, preferably any amino acid that does not disrupt the structural fold of the remaining conserved amino acids
  MISC_FEATURE (17)..(17): Xaa corresponds to position 263 of SEQ ID NO:1 and is any amino acid, preferably any amino acid that does not disrupt the structural fold of the remaining conserved amino acids
XXYCPXXXXXPPPEYXXC

SEQ ID NO: 3 - protein, 474 aa, Ovaloparmena affinis
MVRYLAGAVLLLVVLSVAAAVSGARDGDYLHLPSEVSRFFRPQETNDDHGEDSVGTRWAVLIAGSKGYANYRHQAGVCHAYQILKRGGLKDENIVVFMYDDIAYNESNPRPGVIINSPHGSDVYAGVPKDYTGEEVNAKNFLAAILGNKSAITGGSGKVVDSGPNDHIFIYYTDHGAAGVIGMPSKPYLYADELNDALKKKHASGTYKSLVFYLEACESGSMFEGILPEDLNIYALTSTNTTESSWCYYCPAQENPPPPEYNVCLGDLFSVAWLEDSDVQNSWYETLNQQYHHVDKRISHASHATQYGNLKLGEEGLFVYMGSNPANDNYTSLDGNALTPSSIVVNQRDADLLHLWEKFRKAPEGSARKEEAQTQIFKAMSHRVHIDSSIKLIGKLLFGIEKCTEILNAVRPAGQPLVDDWACLRSLVGTFETHCGSLSEYGMRHTRTIANICNAGISEEQMAEAASQACASIP

SEQ ID NO: 4 - protein, 462 aa, Clitoria ternatea
IRDDFLRLPSQASKFFQADDNVEGTRWAVLVAGSKGYVNYRHQADVCHAYQILKKGGLKDENIIVFMYDDIAYNESNPHPGVIINHPYGSDVYKGVPKDYVGEDINPPNFYAVLLANKSALTGTGSGKVLDSGPNDHVFIYYTDHGGAGVLGMPSKPYIAASDLNDVLKKKHASGTYKSIVFYVESCESGSMFDGLLPEDHNIYVMGASDTGESSWVTYCPLQHPSPPPEYDVCVGDLFSVAWLEDCDVHNLQTETFQQQYEVVKNKTIVALIEDGTHVVQYGDVGLSKQTLFVYMGTDPANDNNTFTDKNSLGTPRKAVSQRDADLIHYWEKYRRAPEGSSRKAEAKKQLREVMAHRMHIDNSVKHIGKLLFGIEKGHKMLNNVRPAGLPVVDDWDCFKTLIRTFETHCGSLSEYGMKHMRSFANLCNAGIRKEQMAEASAQACVSIPDNPWSSLHAGFSV

SEQ ID NO: 5 - protein, 488 aa, Coffea canephora
MMRYATAALLLLALSIIAVAEARDNFLKLPSEIADFFHPKERSDAGGDSVGTRWAVLIAGSNGYWNYRHQADVCHAYQILKRGGLKDENIVVFMYDDIAYNEENPRPGVIINSPHGADVYQGVPKDYTGDDVNAKNFLAAILGDKTAITGGSGKVVDSGPNDHIFIYYTDHGGPGVLGTPSGPYLYADDLNEVLKKKHASGTYKSLVFYLEACESGSIFEGLLPEDLNIYATTASNAEESSWGTYCPGEYPSPPPEYETCLGDLYSVAWMEDSEIHNLHTETLKQQYHLVKKRTSSSNSAYGSHVMQYGDLKLSLEDLFLYMGTNPANDNYTFVDENSLRPSSKAVNQRDADLLHFWDKFRKAPEGSARKVEAQKQVVEAMSHRMHIDNSVKLIGKLLFGIEKGSEILNSVRPAGHPLADDWDCLKSLVRTFETHCGSLSQYGMKHMRSIANICNAGIKKDQMAEAAAQACVSLPSNSWSSLHRGFSA

SEQ ID NO: 6 - protein, 491 aa, Daucus carota subsp. sativus
MVRYLAGAVALLVVVSISAVVESRRDIVGDVLKLPSEVSSFFRPVAEEEDSVGTRWAVLIAGSNGYWNYRHQADICHAYQLLRRGGVKEENIVVFMYDDIAYDEENPRPGVIINSPHGSDVYKGVPKDYTGEDVTVNNVFAAILGDKSATTGGSGKVVDSGPNDHIFIYYSDHGGPGVLGMPTNPYMYAGDLVDVLKKKHASGTYKSMVFYLEACESGSIFEGLLPEGLNIYATTASNAYESSWGTYCPGEYPSPPPEYETCLGDLYSVAWMEDSDIHNLRTETLRQQYQQVKKRTSNDNSGWGSHVMQYGDLKLSTEELFMYMGTNPANDNFTFVDDNSLRLSSSKAVNQRDADLLHFWDKYRKAPEGSDRKIAAQKQFSEAMSHRMHLDNSIQLIGKLLFGIDTASEVLTTVRPSGQPLVDDWLCLKKLVRTFETYCGSLSQYGMKHMRSIANICNAGISEEQMSEASAQACVTFPSNPWSSVNKGFTA

SEQ ID NO: 7 - protein, 486 aa, Corchorus capsularis
MTRLVAGVILLLLSVTGIVSAGRDATGDVLRLPSEASRFFRPSDDDEVGTRWAVLIAGSNGYWNYRHQADVCHAYQLLKKGGLKDENIIVFMYDDIAYNYENPRQGIIINSPHGDDVYQGVPKDYTGEEVTVHNFLAAILGNKTAITGGSGKVVDSGPNDHIFIYYTDHGGPGVLGMPTYPYLYADELIDTLKKKHASGTYKSLVFYLEACESGSIFEGLLPEGLNIYATTASNADESSWGTYCPGEYPSPPPEYETCLGDLYSVAWMEDSDLHNLRTETLHQQYELVKRRTLNGNSAYGSHVMQYGDVGLAKEHLFLYLGTNPANDNFTFIDENSLQPPAKAVNQRDADLVHFWDKYRKAPDGSARKVEAQKQVVEAMSHRMHVDNSIQLIGKLLFGIERGADVLKTVRPAGQPLVDDWKCLKSMVRTFETHCGSLAQYGMKHMRSIANICNAGIQTEQIAEASAQACVSIPSGQWSSIQKGFSA

SEQ ID NO: 8 - protein, 486 aa, Corchorus olitorius
MTRLVAGVILLLLSVTGIASAGRDATGDVLRLPSEASRFFRPSDDDEVGTRWAVLIAGSNGYWNYRHQADVCHAYQLLKKGGLKDENIIVFMYDDIAFNYENPRQGIIINSPHGDDVYQDVPKDYTGEEVTVHNFLAAILGNKTAIKGGSGKVVDSGPNDHIFIYYTDHGGPGVLGMPTYPYLYADELIDTLKKKHASGTYKSLVFYLEACESGSIFEGLLPEGLNIYATTASNADESSWGTYCPGEYPSPPPEYETCLGDLYSVAWMEDSDLHNLRTETLHQQYELVKRRTLNGNSAYGSHVMQYGDVGLAKEHLFLYLGTNPANDNFTFIDENSLQPPAKAVNQRDADLVHFWDKYRKAPDGSVRKVEAQKQVVEAMSHRMHVDNSIQLIGKLLFGIERGADVLKTVRPAGQPLVDDWKCLKSMVRTFETHCGSLAQYGMKHMRSIANICNAGIQTEQMAEASSQACVSIPSGQWSSIQKGFSA

SEQ ID NO: 9 - protein, 493 aa, Jatropha curcas
MTRLATGVILLLLALCVVSSAGSRDIVGDVLRLPSEASRFFRPGGAHVAKEDDSTGTRWAILIAGSNGYWNYRHQADVCHAYQLLKKGGLKDENIIVFMYDDIAFNKENPRPGVIINNPYGEDVYKGVPKDYTGEDVNVNNFFAAILGNKTAITGGSGKVVDSGPNDHIFIYYTDHGGPGVLGMPTNPYLYANDLIDVLIKKHASGTYKSLVFYLEACESGSIFEGLLPEGLNIYATTAANAEESSWGTYCPGEYPSPPPEYETCLGDLYSVAWMEDSDVHNLQTETLRQQYQLVKRRTANGNSAYGSHVMQYGDVGLSKDNLFLYMGTNPANENYTFVDENSLRPPSKAVNQRDADLVHFWDKYRKAPDGSTRKIQAQKQFVEAMSHRMHLDHSMKLIGKLLFGIGKGSEVLNAIRPAGQPLVDDWVCLKTLVRTFETHCGSLSQYGMKHMRSLANLCNAGIREDQMAEASAQACVSIPSGPWSSLHKGFSA

SEQ ID NO: 10 - protein, 494 aa, Malus hupehensis
MTRLASAVVLLFLASVLASAAGSRDLIGDVLRLPSEASRFFGRGDDAPDQQDDGTVGTRWAVLIAGSNGYWNYRHQADICHAYQLLKKGGLKDENIVVFMYDDIAYNEENPRQGVIINSPHGSDVYEGVPKDYTGEDVTVNNFFAAILGNKTALTGGSGKVVDSGPNDHIFIYYTDHGGPGILGMPTSPYIYANDLIEVLKKKHAAGTYRSLVFYLEACESGSIFEGLLPEGLNIFATTASNAEESSWGTYCPGEYPSPPPEYDTCLGDLYSVAWMEDSDVHNLRSETLHQQYELVKTRAANDNSGSGSHVMQYGDVGLSKNNLFVYMGTNPANDNYTFLGENSLRPSSKAVNQRDADLLHFWHKYRKAPEGSARKIQAQKDFVEAMSHRMHIDQTMKLIGKLLFGIEKGPQVLNAVRPAGQPLVDDWDCLKTMVRSFETHCGSLSQYGMKHMRSLANICNAGMTQEQMAEASAQACVSAPSGRWSSLHRGFSA

SEQ ID NO: 11 - protein, 494 aa, Pyrus x bretschneideri
MTRFAGAVVLLFLASVLASAAGSRDLIGDVLRLPSEASRFFGRGDDAPDQQDDGTVGTRWAVLIAGSNGYWNYRHQADICHAYQLLKKGGLKDENIVVFMYDDIAYNEENPRQGVIINNPQGSDVYEGVPKDYTGEDVTVNNFFAAILGNKTALTGGSGKVVDSGPNDHIFIYYTDHGGPGVLGMPTSPYIYANDLIEVLKKKHAAGTYKSLVFYLEACESGSIFEGLLPEGLNIFATTASNAEESSWGTYCPGEYPSPPPEYETCLGDLYSVAWMEDSDIHNLRSETLHQQYELVKTRTANDNYGFGSHVMQYGDVGLSKNNLFVYMGTNPANDNYTFLGENSLRPSSKAVNQRDADLLHFWHKYRKAPEGSARKVQAQKDFVEAMSHRMHIDQTMKLIGKLLFGIEKGPQVLNAVRPAGQPLVDDWDCLKTMVRSFETHCGSLSQYGMKHMRSLANICNAGMTQEQMAEASAQACVSAPSSRWSSLHRGFSA

SEQ ID NO: 12 - protein, 537 aa, artificial sequence
  artificial sequence
MGMAHHHHHHMQIFVKTLTGKTITLEVEPSDTIENVKAKIQDKEGIPPDQQRLIFAGKQLEDGRTLSDYNIQKESTLHLVLRLRGGARDGDYLHLPSEVSRFFRPQETNDDHGEDSVGTRWAVLIAGSKGYANYRHQAGVCHAYQILKRGGLKDENIVVFMYDDIAYNESNPRPGVIINSPHGSDVYAGVPKDYTGEEVNAKNFLAAILGNKSAITGGSGKVVDSGPNDHIFIYYTDHGAAGVIGMPSKPYLYADELNDALKKKHASGTYKSLVFYLEACESGSMFEGILPEDLNIYALTSTNTTESSWCYYCPAQENPPPPEYNVCLGDLFSVAWLEDSDVQNSWYETLNQQYHHVDKRISHASHATQYGNLKLGEEGLFVYMGSNPANDNYTSLDGNALTPSSIVVNQRDADLLHLWEKFRKAPEGSARKEEAQTQIFKAMSHRVHIDSSIKLIGKLLFGIEKCTEILNAVRPAGQPLVDDWACLRSLVGTFETHCGSLSEYGMRHTRTIANICNAGISEEQMAEAASQACASIP

SEQ ID NO: 13 - protein, 10 aa, artificial sequence
  artificial sequence
MGMAHHHHHH

SEQ ID NO: 14 - protein, 76 aa, artificial sequence [sequence omitted]

SEQ ID NO: 15 - protein, 450 aa, Ovaloparmena affinis
ARGDYLHLPSEVSRFFRPQETNDDHGEDSVGTRWAVLIAGSKGYANYRHQAGVCHAYQILKRGGLKDENIVVFMYDDIAYNESNPRPGVIINSPHGSDVYAGVPKDYTGEEVNAKNFLAAILGNKSAITGGSGKVVDSGPNDHIFIYYTDHGAAGVIGMPSKPYLYADELNDALKKKHASGTYKSLVFYLEACESGSMFEGILPEDLNIYALTSTNTTESSWCYYCPAQENPPPPEYNVCLGDLFSVAWLEDSDVQNSWYETLNQQYHHVDKRISHASHATQYGNLKLGEEGLFVYMGSNPANDNYTSLDGNALTPSSIVVNQRDADLLHLWEKFRKAPEGSARKEEAQTQIFKAMSHRVHIDSSIKLIGKLLFGIEKCTEILNAVRPAGQPLVDDWACLRSLVGTFETHCGSLSEYGMRHTRTIANICNAGISEEQMAEAASQACASIP

SEQ ID NO: 16 - DNA, 38 bp, artificial sequence
  primer used for mutagenesis
caccaccgaaagcagctgggcctactattgcccggcgc

SEQ ID NO: 17 - protein, 14 aa, artificial sequence
  Peptide template used for characterizing recognition sequence specificity of Quicklase
  MISC_FEATURE (1)..(1): Xaa is any amino acid. In each screen, only one of the residue is modified. The default amino acid at Xaa1 position is Gly, at Xaa2 position is Leu, and at Xaa3 position is Gly, and at the Xaa4 position is Leu, in this screen.
  MISC_FEATURE (2)..(2): Xaa is any amino acid. In each screen, only one of the residue is modified. The default amino acid at Xaa1 position is Gly, at Xaa2 position is Leu, and at Xaa3 position is Gly, and at the Xaa4 position is Leu, in this screen.
  MISC_FEATURE (13)..(13): Xaa is any amino acid. In each screen, only one of the residue is modified. The default amino acid at Xaa1 position is Gly, at Xaa2 position is Leu, and at Xaa3 position is Gly, and at the Xaa4 position is Leu, in this screen.
  MISC_FEATURE (14)..(14): Xaa is any amino acid. In each screen, only one of the residue is modified. The default amino acid at Xaa1 position is Gly, at Xaa2 position is Leu, and at Xaa3 position is Gly, and at the Xaa4 position is Leu, in this screen.
XXYRRGRLYRRNXX